European Patent Application EP 4 737 574 A2, published May 6, 2026. Title: POLY-TAILED AND POLY-CAPPED MRNA AND USES THEREOF. Applicant: THE BROAD INSTITUTE, INC. Application EP, filed January 18, 2023. The sequence listing filed with the application follows.

SEQUENCE LISTING (27 sequences)

SEQ ID NO: 1 - RNA, 34 nt, synthetic construct
  source 1..34: mol_type = other RNA
  modified_base 7: mod_base = OTHER; note = Modified uridine deoxyribonucleotide with an attachment point on the uridine
  modified_base 20: mod_base = OTHER; note = Modified uridine deoxyribonucleotide with an attachment point on the uridine
  modified_base 33: mod_base = OTHER; note = Modified uridine deoxyribonucleotide with an attachment point on the uridine
  modified_base 34: mod_base = OTHER; note = Cytosine dideoxyribonucleotide
aaaaaataaaaaaaaaaaataaaaaaaaaaaatc

SEQ ID NO: 2 - RNA, 30 nt, synthetic construct
  source 1..30: mol_type = other RNA
  modified_base 25..30: mod_base = OTHER; note = Phosphorothioate linkage
aaaaaaaaaaaaaaaaaaaaaaaaaaaaaa

SEQ ID NO: 3 - RNA, 30 nt, synthetic construct; identical to SEQ ID NO: 2
  source 1..30: mol_type = other RNA
  modified_base 25..30: mod_base = OTHER; note = Phosphorothioate linkage

SEQ ID NO: 4 - RNA, 36 nt, synthetic construct
  source 1..36: mol_type = other RNA
  modified_base 7: mod_base = OTHER; note = Modified uridine deoxyribonucleotide with an attachment point on the uridine
  modified_base 25: mod_base = OTHER; note = Modified uridine deoxyribonucleotide with an attachment point on the uridine
  modified_base 35: mod_base = OTHER; note = Modified uridine deoxyribonucleotide with an attachment point on the uridine
gggaaataagagagaaaagaagagtaagaagaaata

SEQ ID NO: 5 - RNA, 20 nt, synthetic construct
  source 1..20: mol_type = other RNA
  modified_base 8: mod_base = OTHER; note = Thymidine ribonucleotide
  modified_base 15..20: mod_base = OTHER; note = Phosphorothioate linkage
gggagactgccaccaaaaaa

SEQ ID NO: 6 - RNA, 20 nt, synthetic construct
  source 1..20: mol_type = other RNA
  modified_base 8: mod_base = OTHER; note = Thymidine ribonucleotide
  modified_base 15..20: mod_base = OTHER; note = Phosphorothioate linkage
gggagactgccaccaaaaaa

SEQ ID NO: 7 - RNA, 34 nt, synthetic construct; identical to SEQ ID NO: 1
  source 1..34: mol_type = other RNA
  modified_base 7: mod_base = OTHER; note = 5prime octadiynyl uracil deoxyribonucleotide
  modified_base 20: mod_base = OTHER; note = 5prime octadiynyl uracil deoxyribonucleotide
  modified_base 33: mod_base = OTHER; note = 5prime octadiynyl uracil deoxyribonucleotide
  modified_base 34: mod_base = OTHER; note = Cytosine dideoxyribonucleotide

SEQ ID NO: 8 - RNA, 30 nt, synthetic construct; identical to SEQ ID NO: 2
  source 1..30: mol_type = other RNA
  modified_base 25..30: mod_base = OTHER; note = Phosphorothioate linkage
  modified_base 1..24: mod_base = OTHER; note = Phosphodiester internucleotide linkage

SEQ ID NO: 9 - RNA, 36 nt, synthetic construct; identical to SEQ ID NO: 4
  source 1..36: mol_type = other RNA
  modified_base 7: mod_base = OTHER; note = 5prime octadiynyl uracil deoxyribonucleotide
  modified_base 25: mod_base = OTHER; note = 5prime octadiynyl uracil deoxyribonucleotide
  modified_base 35: mod_base = OTHER; note = 5prime octadiynyl uracil deoxyribonucleotide

SEQ ID NO: 10 - RNA, 34 nt, synthetic construct; identical to SEQ ID NO: 1
  source 1..34: mol_type = other RNA
  modified_base 7: mod_base = OTHER; note = 5prime octadiynyl uracil deoxyribonucleotide
  modified_base 20: mod_base = OTHER; note = 5prime octadiynyl uracil deoxyribonucleotide
  modified_base 33: mod_base = OTHER; note = 5prime octadiynyl uracil deoxyribonucleotide
  modified_base 34: mod_base = OTHER; note = Cytosine dideoxyribonucleotide
  modified_base 27..33: mod_base = OTHER; note = Phosphorothioate linkage
  modified_base 1..26: mod_base = OTHER; note = Phosphodiester internucleotide linkage

SEQ ID NO: 11 - RNA, 31 nt, synthetic construct
  source 1..31: mol_type = other RNA
  modified_base 25..31: mod_base = OTHER; note = Phosphorothioate linkage
  modified_base 31: mod_base = OTHER; note = Cytosine dideoxyribonucleotide
  modified_base 1..24: mod_base = OTHER; note = Phosphodiester internucleotide linkage
aaaaaaaaaaaaaaaaaaaaaaaaaaaaaac

SEQ ID NO: 12 - RNA, 60 nt, synthetic construct
  source 1..60: mol_type = other RNA
aaaaaaaaaaaaaaaaaaaaaaaaaaaaaaaaaaaaaaaaaaaaaaaaaaaaaaaaaaaa

SEQ ID NO: 13 - DNA, 34 bp, synthetic construct
  source 1..34: mol_type = other DNA
  modified_base 7: mod_base = OTHER; note = 5prime octadiynyl uracil deoxyribonucleotide
  modified_base 20: mod_base = OTHER; note = 5prime octadiynyl uracil deoxyribonucleotide
  modified_base 33: mod_base = OTHER; note = 5prime octadiynyl uracil deoxyribonucleotide
  modified_base 34: mod_base = OTHER; note = Cytosine dideoxyribonucleotide
aaaaaataaaaaaaaaaaataaaaaaaaaaaatc

SEQ ID NO: 14 - RNA, 34 nt, synthetic construct
  source 1..34: mol_type = other RNA
  modified_base 20: mod_base = OTHER; note = 5prime octadiynyl uracil deoxyribonucleotide
  modified_base 34: mod_base = OTHER; note = Cytosine dideoxyribonucleotide
  modified_base 27..33: mod_base = OTHER; note = Phosphorothioate linkage
aaaaaaaaaaaaaaaaaaataaaaaaaaaaaaac

SEQ ID NO: 15 - RNA, 34 nt, synthetic construct
  source 1..34: mol_type = other RNA
  modified_base 7: mod_base = OTHER; note = 5prime octadiynyl uracil deoxyribonucleotide
  modified_base 20: mod_base = OTHER; note = 5prime octadiynyl uracil deoxyribonucleotide
  modified_base 34: mod_base = OTHER; note = Cytosine dideoxyribonucleotide
  modified_base 27..33: mod_base = OTHER; note = Phosphorothioate linkage
aaaaaataaaaaaaaaaaataaaaaaaaaaaaac

SEQ ID NO: 16 - RNA, 31 nt, synthetic construct; identical to SEQ ID NO: 11
  source 1..31: mol_type = other RNA
  modified_base 25: mod_base = OTHER; note = 2prime O methyladenosine
  modified_base 26: mod_base = OTHER; note = 2prime O methyladenosine
  modified_base 27: mod_base = OTHER; note = 2prime O methyladenosine
  modified_base 28: mod_base = OTHER; note = 2prime O methyladenosine
  modified_base 29: mod_base = OTHER; note = 2prime O methyladenosine
  modified_base 30: mod_base = OTHER; note = 2prime O methyladenosine
  modified_base 31: mod_base = OTHER; note = Cytosine dideoxyribonucleotide
  modified_base 25..31: mod_base = OTHER; note = Phosphorothioate linkage

SEQ ID NO: 17 - RNA, 34 nt, synthetic construct; identical to SEQ ID NO: 1
  source 1..34: mol_type = other RNA
  modified_base 7: mod_base = OTHER; note = 5prime octadiynyl uracil deoxyribonucleotide
  modified_base 20: mod_base = OTHER; note = 5prime octadiynyl uracil deoxyribonucleotide
  modified_base 33: mod_base = OTHER; note = 5prime octadiynyl uracil deoxyribonucleotide
  modified_base 27: mod_base = OTHER; note = 2prime O methyladenosine
  modified_base 28: mod_base = OTHER; note = 2prime O methyladenosine
  modified_base 29: mod_base = OTHER; note = 2prime O methyladenosine
  modified_base 30: mod_base = OTHER; note = 2prime O methyladenosine
  modified_base 31: mod_base = OTHER; note = 2prime O methyladenosine
  modified_base 32: mod_base = OTHER; note = 2prime O methyladenosine
  modified_base 34: mod_base = OTHER; note = Cytosine dideoxyribonucleotide
  modified_base 27..33: mod_base = OTHER; note = Phosphorothioate linkage

SEQ ID NO: 18 - RNA, 110 nt, synthetic construct
  source 1..110: mol_type = other RNA
  modified_base 12: mod_base = OTHER; note = 5prime octadiynyl uracil deoxyribonucleotide
agataaactagtattcttctggtccccacagactcagagagaacccgccaccatggtgagcggctggcggctgttcaagaagattagctgaaaaaaaaaaaaaaaaaaaa

SEQ ID NO: 19 - RNA, 110 nt, synthetic construct; identical to SEQ ID NO: 18
  source 1..110: mol_type = other RNA
  modified_base 12: mod_base = OTHER; note = 5prime octadiynyl uracil deoxyribonucleotide

SEQ ID NO: 20 - RNA, 15 nt, synthetic construct
  source 1..15: mol_type = other RNA
agagataaactagta

SEQ ID NO: 21 - RNA, 15 nt, synthetic construct
  source 1..15: mol_type = other RNA
agagataaactagta

SEQ ID NO: 22 - RNA, 12 nt, synthetic construct
  source 1..12: mol_type = other RNA
aaaaaaaaaaaa

SEQ ID NO: 23 - RNA, 11 nt, synthetic construct
  source 1..11: mol_type = other RNA
aaaaaaaaaaa

SEQ ID NO: 24 - RNA, 13 nt, synthetic construct
  source 1..13: mol_type = other RNA
aaaaaaaaaaaaa

SEQ ID NO: 25 - RNA, 32 nt, synthetic construct
  source 1..32: mol_type = other RNA
aaaaaaaaaaaaaaaaaaaaaaaaaaaaaaaa

SEQ ID NO: 26 - RNA, 15 nt, synthetic construct
  source 1..15: mol_type = other RNA
aaaaaaaaaaaaaaa

SEQ ID NO: 27 - RNA, 30 nt, synthetic construct; identical to SEQ ID NO: 2
  source 1..30: mol_type = other RNA
  modified_base 25..30: mod_base = OTHER; note = Phosphorothioate linkage